European Patent Specification EP 4 053 270 B1, published August 23, 2023. Title: Novel cytosine permease variant and a method for producing L-tryptophan using the same. Applicant: CJ CheilJedang Corporation. The sequence listing filed with the application follows.

SEQUENCE LISTING (10 sequences)

SEQ ID NO: 1 - protein, 419 aa, Artificial Sequence
  codB
MSQDNNFSQGPVPQSARKGVLALTFVMLGLTFFSASMWTGGTLGTGLSYHDFFLAVLIGNLLLGIYTSFLGYIGAKTGLTTHLLARFSFGVKGSWLPSLLLGGTQVGWFGVGVAMFAIPVGKATGLDINLLIAVSGLLMTVTVFFGISALTVLSVIAVPAIACLGGYSVWLAVNGMGGLDALKAVVPAQPLDFNVALALVVGSFISAGTLTADFVRFGRNAKLAVLVAMVAFFLGNSLMFIFGAAGAAALGMADISDVMIAQGLLLPAIVVLGLNIWTTNDNALYASGLGFANITGMSSKTLSVINGIIGTVCALWLYNNFVGWLTFLSAAIPPVGGVIIADYLMNRRRYEHFATTRMMSVNWVAILAVALGIAAGHWLPGIVPVNAVLGGALSYLILNPTLNRKTTAAMTHVEANSVE

SEQ ID NO: 2 - DNA, 1260 bp, Artificial Sequence
  codB
gtgtcgcaagataacaactttagccaggggccagtcccgcagtcggcgcggaaaggggtattggcattgacgttcgtcatgctgggattaaccttcttttccgccagtatgtggaccggcggcactctcggaaccggtcttagctatcatgatttcttcctcgcagttctcatcggtaatcttctcctcggtatttacacttcatttctcggttacattggcgcaaaaaccggcctgaccactcatcttcttgctcgcttctcgtttggtgttaaaggctcatggctgccttcactgctactgggcggaactcaggttggctggtttggcgtcggtgtggcgatgtttgccattccggtgggtaaggcaaccgggctggatattaatttgctgattgccgtttccggtttactgatgaccgtcaccgtcttttttggcatttcggcgctgacggttctttcggtgattgcggttccggctatcgcctgcctgggcggttattccgtgtggctggctgttaacggcatgggcggcctggacgcattaaaagcggtcgttcccgcacaaccgttagatttcaatgtcgcgctggcgctggttgtggggtcatttatcagtgcgggtacgctcaccgctgactttgtccggtttggtcgcaatgccaaactggcggtgctggtggcgatggtggcctttttcctcggcaactcgttgatgtttattttcggtgcagcgggcgctgcggcactgggcatggcggatatctctgatgtgatgattgctcagggcctgctgctgcctgcgattgtggtgctggggctgaatatctggaccaccaacgataacgcactctatgcgtcgggtttaggtttcgccaacattaccgggatgtcgagcaaaaccctttcggtaatcaacggtattatcggtacggtctgcgcattatggctgtataacaattttgtcggctggttgaccttcctttcggcagctattcctccagtgggtggcgtgatcatcgccgactatctgatgaaccgtcgccgctatgagcactttgcgaccacgcgtatgatgagtgtcaattgggtggcgattctggcggtcgccttggggattgctgcaggccactggttaccgggaattgttccggtcaacgcggtattaggtggcgcgctgagctatctgatccttaacccgactttgaatcgtaaaacgacagcagcaatgacgcatgtggaggctaacagtgtcgaataa

SEQ ID NO: 3 - protein, 419 aa, Unknown
  codB
MSQDNNFSQGPVPQSARKGVLALTFVMLGLTFFSASMWTGGTLGTGLSYHDFFLAVLIGNLLLGIYTSFLGYIGAKTGLTTHLLARFSFGVKGSWLPSLLLGGTQVGWFGVGVAMFAIPVGKATGLDINLLIAVSGLLMTVTVFFGISALTVLSVIAVPAIACLGGYSVWLAVNGMGGLDALKAVVPAQPLDFNVALALVVGSFISAGTLTADFVRFGRNAKLAVLVAMVAFFLGNSLMFIFGAAGAAALGMADISDVMIAQGLLLPAIVVLGLNIWTTNDNALYASGLGFANITGMSSKTLSVINGIIGTVCALWLYNNFVGWLTFLSAAIPPVGGVIIADYLMNRRRYEHFATTRMMSVNWVAILAVALGIAAGHWLPGIVPVNAVLGGALSYLILNPILNRKTTAAMTHVEANSVE

SEQ ID NO: 4 - DNA, 1260 bp, Unknown
  codB
gtgtcgcaagataacaactttagccaggggccagtcccgcagtcggcgcggaaaggggtattggcattgacgttcgtcatgctgggattaaccttcttttccgccagtatgtggaccggcggcactctcggaaccggtcttagctatcatgatttcttcctcgcagttctcatcggtaatcttctcctcggtatttacacttcatttctcggttacattggcgcaaaaaccggcctgaccactcatcttcttgctcgcttctcgtttggtgttaaaggctcatggctgccttcactgctactgggcggaactcaggttggctggtttggcgtcggtgtggcgatgtttgccattccggtgggtaaggcaaccgggctggatattaatttgctgattgccgtttccggtttactgatgaccgtcaccgtcttttttggcatttcggcgctgacggttctttcggtgattgcggttccggctatcgcctgcctgggcggttattccgtgtggctggctgttaacggcatgggcggcctggacgcattaaaagcggtcgttcccgcacaaccgttagatttcaatgtcgcgctggcgctggttgtggggtcatttatcagtgcgggtacgctcaccgctgactttgtccggtttggtcgcaatgccaaactggcggtgctggtggcgatggtggcctttttcctcggcaactcgttgatgtttattttcggtgcagcgggcgctgcggcactgggcatggcggatatctctgatgtgatgattgctcagggcctgctgctgcctgcgattgtggtgctggggctgaatatctggaccaccaacgataacgcactctatgcgtcgggtttaggtttcgccaacattaccgggatgtcgagcaaaaccctttcggtaatcaacggtattatcggtacggtctgcgcattatggctgtataacaattttgtcggctggttgaccttcctttcggcagctattcctccagtgggtggcgtgatcatcgccgactatctgatgaaccgtcgccgctatgagcactttgcgaccacgcgtatgatgagtgtcaattgggtggcgattctggcggtcgccttggggattgctgcaggccactggttaccgggaattgttccggtcaacgcggtattaggtggcgcgctgagctatctgatccttaacccgattttgaatcgtaaaacgacagcagcaatgacgcatgtggaggctaacagtgtcgaataa

SEQ ID NO: 5 - DNA, 40 bp, Artificial Sequence
  Forward Primer
ggaattcgagctcggtacccgctcagggcctgctgctgcc

SEQ ID NO: 6 - DNA, 21 bp, Artificial Sequence
  Reverse Primer
acgattcaaagtcgggttaag

SEQ ID NO: 7 - DNA, 21 bp, Artificial Sequence
  Forward Primer
cttaacccgactttgaatcgt

SEQ ID NO: 8 - DNA, 40 bp, Artificial Sequence
  Reverse Primer
gttatccctagcggatccccgcgcagttagcgttgcatcc

SEQ ID NO: 9 - DNA, 20 bp, Artificial Sequence
  Forward Primer
cctcggcaactcgttgatgt

SEQ ID NO: 10 - DNA, 20 bp, Artificial Sequence
  Reverse Primer
cttcctgcttcacttccagc